European Patent Specification EP 3 388 507 B1, published February 19, 2025. Title: Fabric Softener Compositions. Applicant: The Procter & Gamble Company. The sequence listing filed with the application follows.

SEQUENCE LISTING (115 sequences)

SEQ ID NO: 1 - protein, 109 aa, Bacillus licheniformis
ARYDDVLYFPASRYPETGAHISDAIKAGHADVCTIERSGADKRRQESLKGIPTKPGFDRDEWPMAMCEEGGKGASVRYVSSSDNRGAGSWVGNRLNGYADGTRILFIVQ

SEQ ID NO: 2 - protein, 109 aa, Bacillus subtilis
ASSYDKVLYFPLSRYPETGSHIRDAIAEGHPDICTIDDGADKRREESLKGIPTKPGYDRDEWPMAVCEEGGAGADVRYVTPSDNRGAGSWVGNQMSSYPDGTRVLFIVQ

SEQ ID NO: 3 - protein, 109 aa, Bacillus licheniformis
ARYDDILYFPASRYPETGAHISDAIKAGHSDVCTIERSGADKRRQESLKGIPTKPGFDRDEWPMAMCEEGGKGASVRYVSSSDNRGAGSWVGNRLSGFADGTRILFIVQ

SEQ ID NO: 4 - protein, 245 aa, Serratia marcescens
DTLESIDNCAVGCPTGGSSNVSIVRHAYTLNNNSTTKFANWVAYHITKDTPASGKTRNWKTDPALNPADTLAPADYTGANAALKVDRGHQAPLASLAGVSDWESLNYLSNITPQKSDLNQGAWARLEDQERKLIDRADISSVYTVTGPLYERDMGKLPGTQKAHTIPSAYWKVIFINNSPAVNHYAAFLFDQNTPKGADFCQFRVTVDEIEKRTGLIIWAGLPDDVQASLKSKPGVLPELMGCKN

SEQ ID NO: 5 - protein, 182 aa, Bacillus sp-62451
LPPDLPSKSTTQAQLNSLNVKNEESMSGYSREKFPHWISQGDGCDTRQVILKRDADNYSGNCPVTSGKWYSYYDGITFNDPSQLDIDHVVPLAEAWRSGASSWSTAKREDFANDLNGPQLIAVSASSNRSKGDQDPSTWQPPRAGANCAYAKMWINTKYNWGLHLQSSEKTALQGMLNSCSY

SEQ ID NO: 6 - protein, 182 aa, Bacillus horikoshii
LPPGTPTKSEAQNQLNSLTVKSEGSMTGYSRDLFPHWSGQGNGCDTRQIVLQRDADYYTGTCPTTSGKWYSYFDGVIVYSPSEIDIDHIVPLAEAWRSGASSWTTEQRRAFANDLNGPQLIAVTASVNRSKGDQDPSTWQPPRAGARCAYAKWWINTKHRWNLHLQSSEKSSLQTMLNGCAY

SEQ ID NO: 7 - protein, 180 aa, Paenibacillus sp-18057
QKPLADAPRQTEHDDYDYELIFPSDDYPETALHILGAIEQGYSDVCTIDRGGAEENRKQSLAGIETRSGYDRDEWPMAMCEEGGAGASVAYIDASDNRGAGSWVGHQLSAYEDGTKILFIVEKPKVLFPNQPATAAPAGNNEVRYPNCAAVREAGKAPLRKGDPGYSAKLDRDGDGVACE

SEQ ID NO: 8 - protein, 182 aa, Bacillus sp-62520
LPPGTPSKSEAQSQLNALTVKPEDPMTGYSRDHFPHWISQGNGCNTRQIVLQRDADYYSGACPVTTGKWYSYFDGVIVYSPSEIDIDHIVPLAEAWRSGASSWTTEKRRSFANDLNGPQLIAVTASVNRSKGDQDPSTWQPPRAGARCAYAKWWINTKHRWGLHLQSSEKSSLQSMLNGCAY

SEQ ID NO: 9 - protein, 182 aa, Bacillus sp-62520
LPPGTPSKSEAQSQLNALTVKPEDPMTGYSRDHFPHWISQGNGCNTRQIVLQRDADYYSGACPVTTGKWYSYFDGVIVYSPSEIDIDHIVPLAEAWRSGASSWTTEQRRSFANDLNGPQLIAVTASVNRSKGDQDPSTWQPPRAGARCAYAKWWINTKHRWGLHLQSSEKSSLQSMLNGCAY

SEQ ID NO: 10 - protein, 182 aa, Bacillus horikoshii
LPPGTPSKSEAQSQLNSLTVKSEDPMTGYSRDHFPHWSGQGNGCDTRQIVLQRDADYYSGNCPVTSGKWYSYFDGVIVYSPSEIDIDHVVPLAEAWRSGASSWTTEQRRSFANDLNGPQLIAVTASVNRSKGDQDPSTWQPPRAGARCAYAKWWINTKHRWNLHLQSSEKSALQTMLNGCVY

SEQ ID NO: 11 - protein, 182 aa, Bacillus horikoshii
LPPGTPSKSEAQSQLNSLTVKTEDPMTGYSRDLFPHWSGQGSGCDTRQIVLQRDADYFTGTCPTTSGKWYSYFDGVIVYSPSEIDVDHIVPLAEAWRSGASSWTTEQRRAFANDLTGPQLIAVTASVNRSKGDQDPSTWQPPRAGARCAYAKWWINTKHRWNLHLQSSEKSSLQTMLNGCAY

SEQ ID NO: 12 - protein, 182 aa, Bacillus sp-16840
LPPGTPSKSEAQSQLNALTVKAEDPMTGYSRNLFPHWNSQGNGCNTRQLVLQRDADYYSGNCPVTSGRWYSYFDGVVVTSPSEIDIDHIVPLAEAWRSGASSWTTEKRKEFANDLNGPQLIAVTASVNRSKGDQDPSTWQPPRAAARCGYAKWWINTKYRWDLSLQSSEKSSLQTMLNTCSY

SEQ ID NO: 13 - protein, 182 aa, Bacillus sp-16840
LPPGTPSKSQAQSQLNALTVKAEDPMTGYSRNLFPHWSSQGNGCNTRQLVLQRDADYYSGNCPVTSGRWYSYFDGVVVTSPSEIDIDHIVPLAEAWRSGASSWTTEKRREFANDLNGPQLIAVTASVNRSKGDQDPSTWQPPRVAARCGYAKWWINTKYRWDLSLQSSEKSSLQTMLNTCSY

SEQ ID NO: 14 - protein, 182 aa, Bacillus sp-62668
LPPGTPSKSEAQSQLTSLTVKPEDPMTGYSRDHFPHWISQGNGCNTRQIVLQRDADYYSGNCPVTTGKWYSYFDGVIVYSPSEIDIDHIVPLAEAWRSGASSWTAEQRRNFANDLNGPQLIAVTASVNRSKGDQDPSTWQPPRTGARCAYAKWWINTKYRWGLHLQSSEKSSLQSMLNGCAY

SEQ ID NO: 15 - protein, 185 aa, Bacillus sp-13395
ASAFPPGTPSKSTAQSQLNSLPVKSEGSMNGYSRDKFPHWISQGDGCDTRQLVLKRDGDYYSGSCPVTSGKWYSYYDGITVYSPSEIDIDHIVPLAEAWRSGASGWTTEKRQSFANDLNGPQLIAVTASVNRSKGDQDPSTWQPPRSGSHCAYAKMWVNTKYRWGLHLQSAEKSALQSMLNACSY

SEQ ID NO: 16 - protein, 185 aa, Bacillus horneckiae
ASAFPPGTPSKSTAQSQLNSLTVKSEGSMTGYSRDKFPHWISQGDGCDTRQLVLKRDGDYYSGNCPVTSGKWYSYYDGITVYSPSEIDIDHIVPLAEAWRSGASGWTTEKRQSFANDLNGPQLIAVTASVNRSKGDQDPSTWQPPRSGSHCAYAKMWVNTKYRWGLHVQSAEKSALQSMLNACSY

SEQ ID NO: 17 - protein, 182 aa, Bacillus sp-11238
FPPEIPSKSTAQSQLNSLTVKSEDAMTGYSRDKFPHWISQGDGCDTRQMVLKRDADYYSGSCPVTSGKWYSYYDGITVYSPSEIDIDHIVPLAEAWRSGASSWTTEKRRNFANDLNGPQLIAVTASVNRSKGDQDPSTWQPPRSGARCAYAKMWVNTKYRWGLHLQSAEKSGLESMLNTCSY

SEQ ID NO: 18 - protein, 182 aa, Bacillus cibi [sequence omitted]

SEQ ID NO: 19 - protein, 182 aa, Bacillus sp-18318
FPPGTPSKSTAQSQLNSLTVKSEGSMTGYSRDKFPHWIGQGSGCDTRQLVLQRDADYYSGSCPVTSGKWYSYYDGVTFYDPSDLDIDHVVPLAEAWRSGASSWSTQKRKDFANDLSGPQLIAVSASSNRSKGDQDPSTWQPTRSGAACGYSKWWISTKHKWGLSLQSSEKNALQGMLNSCVY

SEQ ID NO: 20 - protein, 182 aa, Bacillus idriensis
LPPGTPSKSTAQSQLNALTVQTEGSMTGYSRDKFPHWISQGNGCDTRQVVLQRDADYYSGTCPVTSGKWYSYYDGVTLYNPSDLDIDHVVALAEAWRSGASSWTTDKREDFANDLSGTQLIAVSASTNRSKGDQDPSTWQPPRSGAACGYAKWWISTKYKWNLNLQSSEKTALQSMLNSCSY

SEQ ID NO: 21 - protein, 182 aa, Bacillus algicola
FPPGTPSKSEAQSQLNSLTVQSEGSMSGYSRDKFPHWIGQGNGCDTRQLVLQRDADYYSGDCPVTSGKWYSYFDGVTVYDPSDLDIDHMVPMAEAWRSGASSWSTQKREDFANDLSGPHLIAVTASSNRSKGDQDPSTWKPTRYGAHCGYAKWWINTKYVYDLTLQSSEKTELQSMLNTCSY

SEQ ID NO: 22 - protein, 182 aa, Xanthan alkaline community J
LPPNIPSKADALTKLNALTVQTEGPMTGYSRDLFPHWSSQGNGCNTRHVVLKRDADSVVDTCPVTTGRWYSYYDGLVFTSASDIDIDHVVPLAEAWRSGASSWTSTKRQSFANDLNGPQLIAVSATSNRSKGDQDPSTWQPPRAGARCAYAKMWVETKSRWGLTLQSSEKAALQTAINACSY

SEQ ID NO: 23 - protein, 182 aa, Bacillus vietnamensis
FPPGTPSKSTAQSQLNALTVKSESSMTGYSRDKFPHWIGQRNGCDTRQLVLQRDADSYSGSCPVTSGSWYSYYDGVTFTDPSDLDIDHVVPLAEAWRSGASSWTTAKREDFANDLSGPQLIAVSASSNRSKGDQDPSTWQPPRSGAACGYSKWWISTKYKWGLSLQSSEKTALQGMLNSCIY

SEQ ID NO: 24 - protein, 182 aa, Bacillus hwajinpoensis
IPPGTPSKSAAQSQLDSLAVQSEGSMSGYSRDKFPHWIGQGNGCDTRQLVLQRDADYYSGDCPVTSGKWYSYFDGVQVYDPSYLDIDHMVPLAEAWRSGASSWSTQKREDFANDLDGPHLIAVTASSNRSKGDQDPSTWKPTRYSAHCGYAKWWINTKYVYDLNLQSSEKSALQSMLNTCSY

SEQ ID NO: 25 - protein, 182 aa, Paenibacillus mucilaginosus
LPPGTPSKSTAQSQLNSLTVKSESTMTGYSRDKFPHWTSQGGGCDTRQVVLKRDADYYSGSCPVTSGKWYSYYDGITVYSPSEIDIDHIVPLAEAWRSGASSWTTEKRQNFANDLGGPQLIAVTASSNRAKGDQDPSTWKPTRSGAHCAYAKWWINTKYRWGLHLQSSEKTALQSMLNTCSY

SEQ ID NO: 26 - protein, 182 aa, Paenibacillus mucilaginosus
TPPGTPSKSTAQTQLNALTVKTEGSMTGYSRDLFPHWISQGSGCDTRQVVLKRDADYYSGSCPVTSGKWYSYYDGVTFYDPSDLDIDHIVPLAEAWRSGASSWTTSKRQDFANDLSGPQLIAVSASTNRSKGDQDPSTWQPPRAGAACGYSKWWISTKYKWGLSLQSSEKTALQGMLNSCSY

SEQ ID NO: 27 - protein, 182 aa, Bacillus marisflavi
TPPVTPSKATSQSQLNGLTVKTEGAMTGYSRDKFPHWSSQGGGCDTRQVVLKRDADSYSGNCPVTSGSWYSYYDGVKFTNPSDLDIDHIVPLAEAWRSGASSWTTAQREAFANDLSGSQLIAVSASSNRSKGDQDPSTWQPPRAGAKCGYAKWWISTKSKWNLSLQSSEKTALQGMLNSCVY

SEQ ID NO: 28 - protein, 184 aa, Bacillus luciferensis
ASLPPGIPSLSTAQSQLNSLTVKSEGSLTGYSRDVFPHWISQGSGCDTRQVVLKRDADYYSGNCPVTSGKWYSYYDGVTVYSPSEIDIDHVVPLAEAWRSGASSWTTEKRQNFANDLNGPQLIAVTASSNRSKGDQDPSTWQPTRTGARCAYAKMWINTKYRWGLHLQSSEKSALQSMLNTCSY

SEQ ID NO: 29 - protein, 182 aa, Bacillus marisflavi
TPPVTPSKETSQSQLNGLTVKTEGAMTGYSRDKFPHWSSQGGGCDTRQVVLKRDADSYSGNCPVTSGSWYSYYDGVKFTHPSDLDIDHIVPLAEAWRSGASSWTTAQREAFANDLSGSQLIAVSASSNRSKGDQDPSTWQPPRAGAKCGYAKWWISTKSKWNLSLQSSEKTALQGMLNSCVY

SEQ ID NO: 30 - protein, 182 aa, Bacillus sp. SA2-6
LPSGIPSKSTAQSQLNSLTVKSEGSMTGYSRDKFPHWISQGGGCDTRQVVLKRDADYYSGNCPVTSGKWYSYYDGISVYSPSEIDIDHVVPLAEAWRSGASSWTTTKRQNFANDLNGPQLIAVTASVNRSKGDQDPSTWQPPRYGARCAYAKMWINTKYRWDLNLQSSEKSSLQSMLDTCSY

SEQ ID NO: 31 - protein, 191 aa, Pyrenochaetopsis sp.
LPSPLLIARSPPNIPSATTAKTQLAGLTVAPQGPQTGYSRDLFPHWITQSGTCNTREVVLKRDGTNVVTNSACASTSGSWLSPYDGKTWDSASDIQIDHLVPLSNAWKSGAAAWTTAQRQAFANDLTHPQLVAVTGSVNESKGDDGPEDWKPPLASYYCTYASMWTAVKSNYKLTITSAEKSALTSMLATC

SEQ ID NO: 32 - protein, 190 aa, Vibrissea flavovirens
TPLPIIARTPPNIPTTATAKSQLAALTVAAAGPQTGYSRDLFPTWITISGTCNTRETVLKRDGTNVVVDSACVATSGSWYSPYDGATWTAASDVDIDHMVPLSNAWKSGASAWTTAQRQTFANDLTNPQLLAVTDNVNQAKGDSGPEDWKPSLTSYWCTYAKMWVKVKTVYDLTITSAEKTALTTMLNTC

SEQ ID NO: 33 - protein, 192 aa, Setosphaeria rostrata
APTSSPLVARAPPNVPSKAEATSQLAGLTVAPQGPQTGYSRDLFPHWITQSGTCNTRETVLKRDGTNVVTNSACASTSGSWFSPYDGATWTAASDVDIDHMVPLSNAWKSGAASWTTARRQAFANDLTNPQLLAVTDNVNQAKGDKGPEDWKPPLTSYYCTYSKMWIKVKSVWGLTITSAEKSALTSMLATC

SEQ ID NO: 34 - protein, 192 aa, Endophragmiella valdina
APVPGHLMPRAPPNVPTTAAAKTALAGLTVQAQGSQTGYSRDLFPHWITQSGTCNTREVVLKRDGTNVVTDSACAATSGTWVSPYDGATWTAASDVDIDHMVPLSNAWKSGAASWTTAQRQAFANDLTNPQLLAVTDNVNQSKGDKGPEDWKPPLTSYYCTYAKMWVKVKSVYSLTITSAEKTALTSMLNTC

SEQ ID NO: 35 - protein, 190 aa, Corynespora cassiicola
LPAPLVPRAPPGIPTTSAARSQLAGLTVAAQGPQTGYSRDLFPHWITQSGSCNTREVVLARDGTGVVQDSSCAATSGTWRSPFDGATWTAASDVDIDHMVPLSNAWKSGAASWTTSRRQAFANDLTNPQLIAVTDNVNQSKGDKGPEDWKPPLTSYYCTYAKMWVRVKSVYSLTITSAEKSALTSMLDTC

SEQ ID NO: 36 - protein, 192 aa, Paraphoma sp. XZ1965
APAPVHLVARAPPNVPTAAQAQTQLAGLTVAAQGPQTGYSRDLFPHWITQSGACNTRETVLKRDGTGVVQDSACAATSGTWKSPYDGATWTAASDVDIDHMVPLSNAWKSGAASWTTARRQAFANDLTNPQLLAVTDNVNQAKGDKGPEDWKPPLTSYYCIYARMWIKVKSVYSLTITSAEKSALTSMLGTC

SEQ ID NO: 37 - protein, 186 aa, Monilinia fructicola
TPVPAPTGIPSTSVANTQLAALTVAAAGSQDGYSRDLFPHWITISGACNTRETVLKRDGTNVVVNSACAATSGTWVSPYDGATWTAASDVDIDHLVPLSNAWKAGASSWTTAQRQAFANDLVNPQLLAVTDSVNQGKSDSGPEAWKPSLKSYWCTYAKMWIKVKYVYDLTITSAEKSALVTMMDTC

SEQ ID NO: 38 - protein, 190 aa, Curvularia lunata
APAPLSARAPPNIPSKADATSQLAGLTVAAQGPQTGYSRDLFPHWITQSGTCNTRETVLKRDGTNVVTSSSCAATSGTWFSPYDGATWTAASDVDIDHVVPLSNAWKSGAASWTTARRQAFANDLTNPQLIAVTDSVNQAKGDKGPEDWKPPLSSYYCTYSKMWIKVKSVYGLTVTSAEKSALSSMLATC

SEQ ID NO: 39 - protein, 191 aa, Penicillium reticulisporum
LPAPEALPAPPGVPSASTAQSELAALTVAAQGSQDGYSRSKFPHWITQSGSCDTRDVVLKRDGTNVVQSASGCTITSGKWVSPYDGATWTASSDVDIDHLVPLSNAWKSGASGWTTAARQAFANDLTNPQLLVVTDNVNESKGDKGPEEWKPPLTSYYCTYAEMWVKVKSVYKLTITSAEKSALTSMLSTC

SEQ ID NO: 40 - protein, 191 aa, Penicillium quercetorum
LPAPEPAPSPPGIPSASTARSELASLTVAPQGSQDGYSRAKFPHWIKQSGSCDTRDVVLERDGTNVVQSSTGCTITGGTWVSPYDGATWTASSDVDIDHLVPLSNAWKSGASAWTTAQRQAFANDLTNPQLVAVTDNVNEAKGDKGPEEWKPPLTSYYCTYAEMWVKVKSVYKLTITSAEKSALSSMLNTC

SEQ ID NO: 41 - protein, 192 aa, Setophaeosphaeria sp.
LPAPVTLEARAPPNIPSTASANTLLAGLTVAAQGSQTGYSRDLFPHWITQSGTCNTRETVLKRDGTGVVTDSACASTSGSWYSVYDGATWTAASDVDIDHVVPLSNAWKSGAASWTTARRQSFANDLTNPQLIAVTDNVNQAKGDKGPEDWKPPLTSYYCTYAKMWVKVKSVYSLTITSAEKTALTSMLNTC

SEQ ID NO: 42 - protein, 192 aa, Alternaria sp. XZ2545
LPAPVTLEARAPPNIPTTAAAKTQLAGLTVAAQGPQTGYSRDLFPHWITQSGTCNTRETVLKRDGTGVVTDSACASTSGSWFSVYDGATWTAASDVDIDHVVPLSNAWKSGAASWTTARRQSFANDLTNPQLIAVTDNVNQAKGDKGPEDWKPPLTSYYCTYAKMWVKVKSVYALTITSAEKTALTSMLNTC

SEQ ID NO: 43 - protein, 192 aa, Alternaria sp.
LPAPVTLEARAPPNIPTTAAAKTQLAGLTVAAQGPQTGYSRDLFPHWITQSGSCNTREVVLQRDGTGVVTDSACAATSGSWYSVYDGATWTAASDVDIDHMVPLSNAWKSGAASWTTARRQAFANDLTNPQLLAVTDNVNQAKGDKGPEDWKPPLTSYYCTYAKMWVKVKSVYALTITSAEKTALTSMLNTC

SEQ ID NO: 44 - protein, 186 aa, Trichoderma reesei
APLPAPPGIPSEDTARTQLAGLTVAVVGSGTGYSRDLFPTWDAISGNCNAREYVLKRDGEGVQVNNACEAQSGSWISPYDNASFTNASSLDIDHMVPLKNAWISGASTWTTAQREALANDVSRPQLWAVSASSNRSKGDRSPDQWKPPLTSFYCTYAKSWIDVKSYYKLTITSAEKTALSSMLDTC

SEQ ID NO: 45 - protein, 188 aa, Chaetomium thermophilum
APAPQPTPPGIPSRSTAQSYLNSLTVAASYDDGNYNRDLFPHWNTVSGTCNTREYVLKRDGSNVVTNSACQATSGTWYSPYDGATWTAASDIDIDHMVPLKNAWISGANTWSSSKRSSFANDINSPQLWAVTDSVNQSKGDKSPDKWKPPLTTFYCTYAKSWITVKYNYNLTITSAEKSALQNMINTC

SEQ ID NO: 46 - protein, 190 aa, Scytalidium thermophilum
LPAPAPMPTPPGIPSKSTAQSQLNALTVKASYDDGKYKRDLFPHWNTVSGTCNTREYVLKRDGVNVVTNSACAATSGTWYSPFDGATWTAASDVDIDHMVPLKNAWISGANNWTSTKRTQFANDINLPQLWAVTDDVNQAKGDKSPDKWKPPLTSFYCTYAKSWITVKYNYGLSITSAEKSALTSMINTC

SEQ ID NO: 47 - protein, 186 aa, Metapochonia suchlasporia
VPVPAPPGIPSTSTAKTLLAGLKVAVPLSGDGYSREKFPLWETIQGTCNAREFVLKRDGTDVKTNNACVAESGNWVSPYDGVKFTAARDLDIDHMVPLKNAWISGASQWTTERRKALANDITRPQLWAVSAHANRGKSDDSPDEWKPPLKTFWCTYAKSWVQVKSFYELTITDAEKGALAGMLDSC

SEQ ID NO: 48 - protein, 198 aa, Daldinia fissa
APAPIPVAEPAPMPMPTPPGIPSASSAKSQLASLTVKAAVDDGGYQRDLFPTWDTITGTCNTREYVLKRDGANVQVGSDCYPTSGTWTSPYDGGKWTSPSDVDIDHMVPLKNAWVSGANKWTTAKREQFANDVDRPQLWAVTDNVNSSKGDKSPDTWKPPLTSFYCTYASAYVAVKSYWGLTITSAEKSALSDMLGTC

SEQ ID NO: 49 - protein, 188 aa, Acremonium sp. XZ2007
LPLQSRDPPGIPSTATAKSLLNGLTVKAWSNEGTYDRDLFPHWQTIEGTCNAREYVLKRDGQNVVVNSACTAQSGTWKSVYDGETTNSASDLDIDHMIPLKNAWISGAATWTTAQRTSFANDISSPQLWAVTAGVNRSKSDRSPDTWVPPLASFHCTYGKAWVQVKSKWALSITSAEKSALTGLLNKC

SEQ ID NO: 50 - protein, 182 aa, Acremonium dichromosporum
IPPGIPSEATARSLLSSLTVAPTVDDGTYDRDLFPHWSSVEGNCNAREFVLRRDGDGVSVGNDCYPTAGTWTCPYDGKRHSVPSDVSIDHMVPLHNAWMTGASEWTTAEREAFANDIDGPQLWAVTSTTNSQKGSDAPDEWQPPQTSIHCKYAAAWIQVKSTYDLTVSSAEQAALEEMLGRC

SEQ ID NO: 51 - protein, 188 aa, Sarocladium sp. XZ2014
VPIPLPDPPGIPSSSTANTLLAGLTVRASSNEDTYNRDLFPHWVAISGNCNAREYVLRRDGTNVVVNTACVPQSGTWRSPYDGESTTNASDLDIDHMVPLKNAWISGAASWTTAKRQDFANDVSGPQLWAVTAGVNRSKGDKSPDSWVPPLASFHCTYARSWIQVKSSWALSVTSAEKAALTDLLSTC

SEQ ID NO: 52 - protein, 186 aa, Metarhizium sp. HNA15-2
VPVPAPPGIPTASTARTLLAGLKVATPLSGDGYSRTLFPTWETIEGTCNAREFVLKRDGTDVQTNTACVAQSGNWVSPYDGVAFTAASDLDIDHMVPLKNAWISGASQWTTDKRKGLANDITRPQLWAVSAHANRAKGDSSPDEWKPPLKTFWCTYARSWVQVKSYYALTITDAEKGALSGMLDSC

SEQ ID NO: 53 - protein, 188 aa, Acremonium sp. XZ2414
APIAVRDPPGIPSASTANTLLAGLTVRASSNEDSYDRNLFPHWSAISGNCNAREFVLERDGTNVVVNNACVAQSGTWRSPYDGETTGNASDLDIDHMVPLKNAWISGASSWSTTRRQEFANDVSGPQLWAVTAGVNRSKGDRSPDSWVPPLASFHCTYAKSWVQVKSSWSLSVTSAEKAALSDLLGTC

SEQ ID NO: 54 - protein, 186 aa, Isaria tenuipes
APVPEPPGIPSTSTAQSDLNSLQVAASGSGDGYSRAEFPHWVSVEGSCDSREYVLKRDGQDVQADSSCKITSGTWVSPYDATTWTNSSKVDIDHLVPLKNAWISGASSWTKAQRQDFANDIKRPQLYAVSENANRSKGDRSPDGWKPPLKSFYCTYAKSWVAVKSYYKLTITSAEKSALGDMLDTC

SEQ ID NO: 55 - protein, 184 aa, Scytalidium circinatum
APPGIPSASTASSLLGELAVAEPVDDGSYDRDLFPHWEPIPGETACSAREYVLRRDGTGVETGSDCYPTSGTWSSPYDGGSWTAPSDVDIDHMVPLKNAWISGASEWTTAEREAFANDIDGPQLWAVTDEVNQSKSDQSPDEWKPPLSSFYCTYACAWIQVKSTYSLSISSAEQAALEDMLGSC

SEQ ID NO: 56 - protein, 186 aa, Metarhizium lepidiotae
VPVPAPPGIPTASTARTLLAGLKVATPLSGDGYSRTLFPTWETIEGTCNAREFVLKRDGTDVQTNTACVAESGNWVSPYDGVSFTAASDLDIDHMVPLKNAWISGASQWTTDKRKDLANDITRPQLWAVSAHANRSKGDSSPDEWKPPLQTFWCTYSKSWIQVKSHYSLTITDAEKGALSGMLDSC

SEQ ID NO: 57 - protein, 226 aa, Thermobispora bispora
LDIADGRPAGGKAAEAATGTSPLANPDGTRPGLAAITSADERAEARALIERLRTKGRGPKTGYEREKFGYAWADSVDGIPFGRNGCDTRNDVLKRDGQRLQFRSGSDCVVISMTLFDPYTGKTIEWTKQNAAEVQIDHVVPLSYSWQMGASRWSDEKRRQLANDPLNLMPVDGATNSRKGDSGPASWLPPRREIRCAYVVRFAQVALKYDLPVTTADKETMLQQCS

SEQ ID NO: 58 - protein, 191 aa, Sporormia fimetaria
LPAPVLEKRTPPNIPSTSTAQSLLSGLTVAPQGSQTGYSRDLFPHWITVSGTCNTRETVLKRDGSNVVTDSACASVSGSWYSTYDGATWTAASDVDIDHVVPLSNAWKSGAASWTTARRQAFANDLTNPQLIAVTDNVNQAKGDQGPESWKPPLTSYYCTYAKMWVKVKSVYSLTVTSAEKSALSSMLGTC

SEQ ID NO: 59 - protein, 193 aa, Pycnidiophora cf.dispera
LPAPAPVLVAREPPNIPSTSSAQSMLSGLTVKAQGPQDGYSRDLFPHWITISGTCNTRETVLKRDGTNVVTNSACASTSGSWYSPYDGATWTAASDVDIDHIVPLSNAWKSGAASWTTSRRQQFANDLTNPQLIAVTDSVNQAKGDKGPEDWKPSRTSYHCTYAKMWIKVKSVYSLTVTSAEKSALTTMLNTC

SEQ ID NO: 60 - protein, 199 aa, Xanthan alkaline community D
DTDPEPVAGSALEALAGLEVKGPGPDTGYERALFGPPWADVDGNGCDTRNDILARDLTDLTFSTRGDVCEVRTGTFDDPYTGETIDFRRGNATSAAVQIDHVVPLLDAWRKGARAWDDETRRQFANDPLNLLASDGPANQSKGARDASAWLPPNHAFRCPYVARQIAVKAAYELSVTPSESEAMARVLADCPAEPLPAG

SEQ ID NO: 61 - protein, 199 aa, Xanthan alkaline community O
DDEPEPARGSALEALARLEVVGPGPDTGYERELFGPAWADVDGNGCDTRNDILARDLTDLTFSTRGEVCEVRTGTFQDPYTGETIDFRRGNATSMAVQIDHVVPLMDAWRKGARAWDDETRRQFANDPLNLLASDGPANQSKGARDASAWLPPNHAFRCPYVARQIAVKTAYELSVTPSESEAMARVLEDCPAEPVPAG

SEQ ID NO: 62 - protein, 186 aa, Clavicipitaceae sp-70249
VPVPAPPGIPSTSTAKTLLAGLKVATPLSGDGYSRDKFPTWETIQGTCNAREFVIKRDGTDVKTNSACVAESGNWVSPYDGVKFTAARDLDIDHMVPLKNAWISGASQWTTEQRKALANDITRPQLWAVSAHANRGKSDDSPDEWKPPLKTFWCTYAKSWVQVKSFYKLTITDTEKGALAGMLDTC

SEQ ID NO: 63 - protein, 187 aa, Westerdykella sp. AS85-2
FPAPASVLEARAPPNIPSASTAQSLLVGLTVQPQGPQDGYSRDLFPHWITISGTCNTRETVLKRDGSNVVTNSACAATSGTWYSPYDGATWTSASDVDIDHLVPLSNAWKSGAASWTTAKRQQFANDLTNPQLLAVTDRVNQAKGDKGPEAWKPSLASYHCTYAKMWVKVKSKDVRLTGNWTKDDGW

SEQ ID NO: 64 - protein, 194 aa, Humicolopsis cephalosporioides
APTPAPVELERRTPPNIPTTASAKSLLAGLTVAAQGPQTGYSRDLFPHWITISGSCNTRETVLKRDGTGVVTDSACASTAGSWYSPYDGATWTAASDVDIDHMVPLSNAWKSGAAQWTTARRQDFANDLTNPQLFAVTDNVNQEKGDKGPEDWKPSLTSYYCTYAKAWVKVKSVWALTITSAEKSALTTMLNTC

SEQ ID NO: 65 - protein, 190 aa, Neosartorya massa
IPAPVALPTPPGIPSAATAESELAALTVAAQGSSSGYSRDLFPHWISQGGSCNTREVVLARDGSGVVKDSNCYPTSGSWYSPYDGATWTQASDVDIDHVVPLANAWRSGASKWTTSQRQAFANDLTNPQLMAVTDNVNQAKGDDGPEAWKPPLTSYYCTYAKMWVRVKYVYDLTITSAEKSALVSMLDTC

SEQ ID NO: 66 - protein, 191 aa, Roussoella intermedia
APTPALLPRAPPNIPSTATAKSQLAALTVAAQGPQDGYSRDLFPHWITQSGSCNTREVVLKRDGTNVVQDSSCAATSGTWVSPFDGATWTAASDVDIDHLVPLSNAWKSGAASWTTARRQSFANDLTNPQLLAVTDEVNQAKGDKGPEAWKPPLASYHCTYAKMWVKVKSTYSLTITSAEKSALTTMLNTC

SEQ ID NO: 67 - protein, 191 aa, Pleosporales
LPTPSLVKRTPPNIPSTTSAKSLLAGLTVAAQGPQDGYSRDLFPHWITISGTCNTRETVLKRDGTNVVTDSACASTSGSWYSTYDGATWTAASDVDIDHVVPLSNAWKSGAASWTTARRQSFANDLTNPQLIAVTDSVNQSKGDKGPESWKPPLTSYHCTYAKMWVKVKDVYSLTVTSAEKSALTTMLNTC

SEQ ID NO: 68 - protein, 192 aa, Phaeosphaeria sp.
LPAPIHLTARAPPNIPSASEARTQLAGLTVAAQGPQDGYSRDLFPHWITQSGTCNTRETVLKRDGTNVVTNSACASTSGSWFSPYDGATWTAASDVDIDHMVPLSNAWKSGAASWTTARRQAFANDLTNPQLLAVTDNVNQAKGDKGPEDWKPPLTSYYCTYARMWVKVKSVYALTVTSAEKSALTSMLGTC

SEQ ID NO: 69 - protein, 189 aa, Didymosphaeria futilis
LPTPNTLEARAPPNIPSTSAAQSQLSALTVAAQGPQTGYSRDLFPHWITQSGTCNTRETVLKRDGTNVLTDSACASTSGSWKSPYDGATWTAASDVDIDHVVPLSNAWKSGAASWTTARRQSFANDLTNPQLIAVTDNVNQAKGDKGPEDWKPPLTSYYCTYAKMWVKVKSVYSLTITSAEKSALTMLA

SEQ ID NO: 70 - protein, 590 aa, Preussia aemulans
LSISEINGPKYLSPYAGQTVSNVAGIVTAKGPSGIWIRSTTPDRDDKTSESIYVFNKTFGANLTVGDSIVIGGKVEEYRSNKDYVYLTEISSPVLESKISSGNAVKPLVIGKDTSKPPTEQFSSLDGGDVFGVPNNVSLVSVANPTLEPKKYGMDFWESLSGELVTVKKPTALSKPSNFGDTWVVGDWKVTGDNKRGGLTQTDKDANPETIIIGSPLDGSSNPLTVKLGDELSEITGVVTYAFGFYRILPTTALKVVKSQQQELPSATSLISSGKCDGLTFGAYNVENLFTGSKHMPNISAHIVTYLKSPDFIFIQEVQDDNGPTNDGVVSANATLTALTEAIVAAGGPQYTFTDIAPSSNQDGGAPGGNIRVAYLYKASLVRLYKPNPGTALDANEVLAGPTLKFNPGRIDPTNEAWTASRKPLVAEWEVISKNGKDGGKFFTVNVHFGSKGGSSSIQGDARPPVNGGIEDRLAQAQLTANFVKAILAKDRNARIITAGDFNEFASVEPMEEYVKVSGLKDLDEVTKIKDVERYTYLFDMNAQQLDHMYISPALEKKAKYEHIHINTWVDRAAQISDHDPSVAKLDVCS

SEQ ID NO: 71 - protein, 589 aa, Colletotrichum circinans
LTIAEINGNKFLSPFKDQSVTNVTGLVLAKGPSGIWIRSTTPDDDDATSEAVYVYGSTVGANLTVGDLITLDGKIQEYRSATNYIYLTELSSPKNVVVVSKGNEVVPLVIGVDTLNPPTEQYTSLDGGDIYAVPNAVANISAVNPVLEPTLYGLDFWESLSGELVTVKNPVSITRPNQYGDTWVLGDWPTTGRNTHGGITMTDKDSNPEAIIIGSPLDGTKNPESKMGDQLTEITGVVTYAFGFYRILPLTAVSIAKNATNDAPPTTLVSRGDCRGITIGDYNVENLAPNSAHLPAVAAHIVDYLKTPDLIFVQEVQDNTGATNNGVVSSNVTLSTLAAAIEAKSGVFYDFVVVDPVDGKDGGAPGGNIRVAYLYKPDVIELWKPNPGGSLDANEVLPGPQLKYNPGRIAPTSSAWDASRKPLVAAWRAIKGPQNKIFFTVNVHFASKGGSSSLHGDLRPPVNGVVNPRIQQAELTGNFIAEILAADPNARIIAAGDFNEFAFVEPLKAFTAKSGLIDLDEAVGIPVEERYTYVYDMNAQELDHMFVSPALAHKNGTKYEHIHINSWELYDDLVSDHDPSVAQFNVCGC

SEQ ID NO: 72 - protein, 281 aa, Preussia aemulans
LSVPRAAPASIDLRPNDLLKSTRGPYGPNGRGRTGSTSATAFNELQLNLCNSGFANCYANGDSIPEGGELIYATGPNVVTINEICSNDVSTLQSYLGEAWPTDYTYSVFMPAIDRRTNQQYKCKNGAQYGSVVLGRVPSATWSGIDAYGGKYSTQDDSNELRIFVCVAARGDHFACTTHLTSKSEPLAMTQCKALMSDAIPYLKSQSGSTTRTVVAGDFNLEYDTGDAENMQKCVPSGWTRKGDGSVQHTIFDNTLKFGSSKKYGLSYTDHDGWLVKMTVG

SEQ ID NO: 73 - protein, 585 aa, Trichurus spiralis
LSIAEINGNRFISPYNGQTVTNVEGLVTAVSSAGFYLRSTKADRDAATSEGLYVYGSNAAKTVTVGDIITVSGKVSEYRSNVDYLYLTELTSPQNITIVSSGAKVKPLVIGKDTYSPPTSKFSSLDEGGLFGVPNNVSRISVANPKLQPKKYGLDFWESIVGELVTIKEAYGVGRPNQYGDVWVRGNWKVTGKNKQGGLTMTDGDANPETIIIGTPLDASKNPTDTKMGDYYGDITGVVSYAFGFYRVLPLTHITPERNSSAAHPPVSFTSKGSCKGITVADYNAENLAPTSTHLPQVVDQIINMLKTPDLLFLQEVQDNSGSKNDGVVSANVTLTTLVDSLFETSGVQYAFAEVEPENLKDGGQPGGNIRVAYLYRPDVVELYKPNQGGSNDANEVLPGPLLKYNPGRIDPANAAWVDSRKPLVAMWRAVKGGKKPFFTVNVHFTSKGGSTSLHGDARPPVNLGVDQRTMQAEVTADFIAQILEEDKKAYVIAAGDFNEFVQVQPLQTFAKKSGLTELDEVAKISMNERYTYLFDMNSEALDHMYVSKGIGKSVKYEHMNLNTWQNYDDQVSDHDPSVARFDLC

SEQ ID NO: 74 - protein, 592 aa, Pyrenochaetopsis sp.
TTIAEINGPAFLSPFKGQTVANVSGIITAKGPDGLWIRSTLPDRDERTSESLYVFGSKFGANLTVGDSIILGGKVQEYRSSKDYIYLTELSSPVLAKKVSSGNKVDALVIGKDTRDPPTEQYSSLDGGDVFAVPNNVSQISVANPELQPKKYGLDFWESLSGELVTVKKPTALTKPNQYGDTWVVGNWKVTGRNDRDGLTLTDKDANPEAIIIGTPLDGTKNPTDTRMGDSVDEITGVITYAFGYYRILPLTAIKVTKSQKPALPKPTKLESKGKCDGITFGDYNVENLAANSSHLPSIAAHIVNYMKSPDVLFVQEIQDDDGPTNDAVVSANLTLSTLVAAISSAGGPTYAFADIDPVDDQDGGEPGGNIRVAYLYKPSLIRLYKPNPGGSLDANAVNDGPTLKYNPGRIDPTNPAWTASRKPLVAQWEVIGKSNAKKLDTFFTVNVHFGSKGGSSSLHGDARPPVNGGVEDRLAQAQLTANFVKDILSKDKDARIITSGDMNEFAFVEPLEQLKDISGLKDLDVEAGIDKLERYTYLFDMNAQQLDHTFVSKAIAKEDPKYEHIHINTWVDYADQISDHDPSVARLSVCA

SEQ ID NO: 75 - protein, 589 aa, Aspergillus sydowii
VTISEINGNTYLSPFKGESVSDVEGLVTAIGEDGFYLRSTTPDSDDATSESIYVYGSSAVSEVTVGDIIALSGEVSEYRSQAAYLYLTEITSPSSIVVKSSGNEVAPVVIGKDRSPPTEVYSGLDGADGDVYALPNNASQISAENPVLKPELYGMDFWESLSGELVSLTGLTIITKPNQYGDVFVRGDWAVSGLNENGGLTMSANDSNPEAIKIGTPLDGTNNSDSSKVGDTVEDVTGVVQWKFGQYMVLPLTALTVTGSNDTVAGPSTLTGDGTCKSLSIGAYNVENLTPTSTHISKIADHIANYLNGPAIMCLQEIQDNNGATDDGTVTANLTLTKLTGLISAAGGPDYNFTEIPPVNNADGGEPGGNIRVAYLYNPSIVRLHNANPGTSADANEVLVSHGPELKFNPGLIDPDSEAWDASRKPLAAAWETVDGENKFFTVNVHLSSKGGGSAIQGDARPPVNGGVEQRTAQAEVIASFVSDILAADANAKILTTGDFNEFSFVSPLETFVEKSGLRELDDVVGIPATERYTYIYDSNHQQLDHMFVSDGLAKNAQLEHVHVNTWLNYDDAASDHDPSVALFDVCEL

SEQ ID NO: 76 - protein, 597 aa, Cladosporium cladosporioides
VTIAAINGDRFLSPLNGTGVQDVAGLVTAKGPNGFWIRSPEPDTHDRTSESVYVFGRNALGNVTVGDLISVDGNVTEYRSSKDYAYLTEIINPRNIRVVSSGNEVKPVVIGSKTSGIIGKRDVQPPREQFSGLDNGDVFAVPNNQSLISQANPRLEPNLYGMDFWESLSGELVTIKGVTALGRQANTFGDQWVRGDWKSSGKNSRGGLTVTDRDSNPESIIIGAPLDGSSNSKETKLGDELEDITGIVTYVFGFYAIFPQTGTKVKRSIDAFPPPSSIVSNGKCSGLTFGQYNIENFAPNNSRVPLIAEHIVDYLNTPSVMFLQEVQDNSGEANDGVVNSNLTLASLSQAISEISGVDYLWVNVDPVNNQDGGAPGGNIQTPYLYNPLQVRLLNANPGGPNDRNEVLPGPTLRFNPGRIDDGVTFSNSRKPIVAHWEMVDGSGTFFTVNNHWTSKGGSTSLQGDARPPVNGGVDRRIRQAEVTGSFIAEILKQDKNAAIIVAGDLNEFATVAPLRRFVEVSGLKDLDVVAKIPELERYSYTFGASQQQLDHVYASAWASRKVGKGDFEHVHVNTWVAEEDVGSDHDPAVARLNVCST

SEQ ID NO: 77 - protein, 600 aa, Rhinocladiella sp.
LTIAEINGNKYLSPYAGQAVTNISGLVTAKGPSGIFIRSTTPDSDPATSESVYVFGSNAGRNVTVGDVITLDGTVTEFRSTSNPTYLFLTEITSPRNVKTVSSGNHVAPLVIGKDTSAPPTQQFSGLDDGDALGVPNNASLISVTNPELKPSEFGMDFWESLSGELVTIKGAKAISKPNNFGDTWVTGDWKVTGRNARGGLTMTKNDSNPEAIIIGTPLDGTRNANGTKLGDSLEDITGVITYGFGFYRILPVTGIKVTGSAQPALPPSTTLKAGKSCRDLTFGSYNVENLSPTKSILPSIASHIANVMKAPSLVFLQEIQDNNGAVNDAVVDANLTLSTLAAEVNRLSGVNYAYVDVDPVDDQDGGEPGGNIRTAYFYDPTVLRLRNPNPGSPTDANEVLQGDVLRGPELKYNPGRIDPTNAAWERSRKPLTAVWETLDGRNKFFTINVHFASKGGSSSVQGDPRPPINGVIDVRTQQAQITAEFIRDILRKDPTSSVIIAGDFNEFAFVQPLEGFSKTSWMQDLDAVAGIKPEERYTYLFDMNCQQLDHMYVSPVLAAKKYIGRVKYEHIHINTWETRAGQISDHDPSVAQLDVCRLF

SEQ ID NO: 78 - protein, 588 aa, Pyronema domesticum
VSIAEINGPAFLSPYAGKSVTDITGLVTAVGPSGFFLRDVASTSSRLRRNQSGSQAVYVFNSAAAKNVTAGDIININSASVVEYQNNQAYIPLTEITNPSAIQIVSKGHEVIPIPLGRNGLQPPTGQFSALDNGDIFGLPNGASKISSTNATLVPTKFGLDFWESLSGEFVGISSPTALGPTSRYGDIWIRGDWEVTGLNSAGGLTITTGTSSDANPETIIIGSPLDGTKNPSVKLGDILNPIQGVITYGFGFYRLLPTTAISIKSARNATTPVTTLKSEKSCKAVTIGQYNVENLSPSSSHLNAIADHIGYNMGSPDLIYVQELQDNSGATNDGITSGNMTLAALAYAIEGISGIQYHWAEVDPEDNLDGGQPGGNIRVAYLYNPSVFSISGTPGTASEATTVQPGPSLSLNPGRIDPQNVAFTNSRKPLVAQFSVEGTQKPFFAINVHSGSKGGSSSLHGDARPPMNGGIEDRIAQHEAIASFIQALKKEDENVNILAAGDFNEFSGVAPMEVFRDLMWDVDEVVDVSKEERYTYNYDMNCQQLDHTLISAGLKEKVSGYQHLHVNTWSEVETSDHDPSVGVYDLC

SEQ ID NO: 79 - protein, 585 aa, Aspergillus niger
VTIPEINGDRYVSSYQGKRVSGLKGLVTAKGSSGFYIRATDADSDSRTSNSIYVYGSSGVSQVTVGDIVTLSGKVTEYRSSSSYVYSTEIESPSDIQVLSSDNIVTPVVIGKDNLDPPTEQYSSLDNGDVFSLPGNSSRLSTANPVLEPTEYGMDFWQSLSGELATLTGLTAISKANSYGDTWVIGDWPVTGKNDRGGLTMRANDSNPESIVIGSPLDGTKNPTDTKLGDTLEDITGIITQAYGFYTLLPLTALTKTGSNTTEATATTLQADGTCSSITIGDYNVDNFSPQSSTMSGIGEHIAKYLNSPTVLFLQEIQDNSGATDDGVVSANETLSKLASAVKEHGGVAYNYTDIDPENDTNGGERGGNIRPAYLFDPSVVRLRNYNPGSSTDSTSVLSDGSLSYNPGLIDPSNEAWDDSRKPLVAQWETLDGKNTFYTINVHFTSKYDSTSLEGDPRPPVNGWVENRVDQAKVVAKFVTSILDVNSDAKIITAGDFNEYAFVEPLEVFVSESKLQDLEEVTGIPATERYTYLYNQNCESLDHMYVSSALTSGAKMEHIHVNSWVSTDDELSDHDPTVALFNMCE

SEQ ID NO: 80 - protein, 587 aa, Phialophora geniculata
ATIAEINGNRFMSPLQGEVVTGVEGLVLAKGPNGIWLRSTVPDDDDLTSEAVYVFDRNIIARLSVGDIVKLDGTILEYRAQAAHMYLTEITATSNLEILSSNNTVTAYVIGEDTGAPPTEQYSSLDEGDIFAVPNNVYRVSEENPVLEPSKYGMDYWRAINGELVTIKTPVGVSRPNQFGDTWVVGTWPTTGRNSQGGLTLRDKDANPEAIIIGSPLDGTRNPETKMGDKFAEITGVVTYAFGFYRILPLTAIEVEEEATIEVSPTTLESRGDCRGLTFASYNIENLWAESEHLPEVAAHIVEYLKTPDFLFLQEVQDNNGPTNNGVVSANITLSNLAAEIEAQSGIVYEFAEVEPVNNQDGGQPGGNIRNAYLYRPDVIELYEPNQGGSTDQAEVVDGPALSFNPGRIDISNSAWDASRKPLVAQWRAVRGPRSKTFFTVNVHNGSKGGSSTLHGDFRPPVNNGVEKRTQQTESVGAFVDAILAQDPKARIIAAGDWNEFQFVQPQRVIAEKHNMTDLSVLALDEIEQYNYVFDMNAQQLDHILVSPALATDAAKIEHLHLAAWLRYPDLTSDHDPLVSYLNVCGC

SEQ ID NO: 81 - protein, 592 aa, Paradendryphiella salina
LSIAEINGPKFLSPYRDQTVSNISGIVTAKGPNGLWLRSPTPDRDERTSESLYVYGSTFGANLTVGDIIVVGGRVTEYQSSKDYIPLTELSAPVLEKKLSSGANVQPLVIGVDTRDPPNKQYSSLDGGDVFAVPNNVSQISVANPALQPKEFGLDFWESLMGELVTVKNPTALTKPNQYGDTWVAGDWKVSGRNKRGGLTMTDKDANPEAIIIGSPLDGTRNPTDTRMGDSVEEITGVVTYAFGFYRILPTTAITVTKSQTPDLPPASTLVSSGTCDGITFGVYNVENLAPSSDHHPDLANHIVNYMNSPDIIFVQEVQDDNGPTNDQVVSANLTLSTLSAAIATAGGPNYAFTEIVPVDDQDGGQPGGNIRNAYLYKPNVLRLYKPNLGGSLDATEVVAGPTLSYNPGRIEPENEAWTNSRKPLAAQWEVIGKRGAKKPNVFFTVNVHFGSKGGSSSLHGDARPPVNGGVDDRLEQALLTANFVKDILSQDKNARIVTAGDFNEFAFVQPLEEYTKISGLKDLDEVVKLDKLERYTYLYDMNTQELDHMFVSPSLAKSRAKFEHIHVNTWPEYDAQVSDHDPSVARLDVCA

SEQ ID NO: 82 - protein, 594 aa, Aspergillus insuetus
AVTIAEINGNAYLSPLKGESVSGVEGLVTAIGESGFFLRSTTPDSDDATSESIYVYGSSSVSKVTVGDIITLSGKVSEYRSQDTYLHLTEITSPSSIVVKSSGNEVTPVVIGKDRSPPTEVYSSLDIGDIYALPNNISRISEENSALKPDVNGLDFWESLSGELVSLTDLTIITKPNQYGDVFVRGNWAVSGLNEHGGLTMTAKDSNPEAIKIGTPLDGTRNRDDSKVGDIVEDVTGVVQWVFGQYMVLPTTALKVTASNDTAAPASTLVGDGTCKSLSIGSYNVENLTPTASNIEGIANHIANYLNGPALVALQEIQDNSGATDDGVVSANVTLSTLANLIAAAGGPDYEFTEIVPVNNADGGQPGGNIRVAYLYDPTIIRLRNENIGSSTDANEVLAGAELKYNPGLIDPSNAAWDASRKPLAAAWETLDGKNKFFTVNVHFSSKGGGTTLQGDVRPPVNGAVDQRIAQAEVVASFIASILEKDPKAKILATGDFNEFAFVEPLTTFVAKSSLVDLDEVVGIPETERYTYIYDSNHQQLDHMFVSEALGKGAKMEHVHVNTWLNYDDASSDHDPSVAVFNVCGKKSTCKPKY

SEQ ID NO: 83 - protein, 588 aa, Purpureocillium lilacinum
VAIAEINGDRFLSPFQDKDVANVTGLVTATSKTGIYLRSTAPDDSPATSEGLFVFSSSLVKTAKVGDVVTLSGLVKEYRSNKDYIYLTELTNPTNVVVVSSGNAVAPLVVGKDTLPPPTRDFSSLDAGGVFGVPNAAGTVSGANPKLDPTAYGLDFWESLVGELVTVKDAYLTSRPNQYGDVWVRGDWAVTGVNGHGGVTMLDGDANPETIVVGTPLDGSANPTDTKMGDFVGDVTGVVSNAFGFYRILPLTRLVPQRNASAEFPATSLASRGSCRGITVADYNAENLAPDSAHLPRVVDQIVNELRLPDLVFLQEVQDNSGAANDGVVSANLTLSTLTRGIEAASGVAYAFAEVEPQDGKDGGQPGGNIRCAYLYRPDVVELHEPRQGGSLDANEVLPGPALKFNPGRIQPANAAFDDSRKPVAAAWRTVKGTHKTFFTVNVHFGSKGGSTTLHGDARPPVNKGVEKRTEQATITADFIAAILKQDPRARVIAAGDFNEFTQVQPMRVFAERSGLRDLDELAGLAPEERYTYLFDMNSQALDHMYVSPALGRGARVEHLHVNTWQNFKGQTSDHDPSVALLNVCGCA

SEQ ID NO: 84 - protein, 586 aa, Warcupiella spinulosa
ITIAEINSNKYLSPYKGQTISGIEGLVTAKGSAGFYLRSTTPDDDDATSESIYVYGSSAVSKVAVGDIITLTGKVAEYRSSSSSYVYLTELTSPSNIVVSSSGNTVTPVVIGQRGLIPPTEQFSALDGGDVFGVPNNDSQISLVNPTLKPEKYGMDFWESLSGELATVKGVRAVSKPNRYGDTWVVGDWKSTGMNERGGLTMTDKDGNPEAIVIGSPLDGSSNPDNTKLGDYLDDITGVITQAYGYYALLPLTALTVRESNSTNATATRLAADGNCSAITVGDYNVNNLSPSSTTLSHIANHIANYLKSPTVMFVQEIQDDNGATNDGVVSANLTLSTLVREIKSAGGIAYSFVDIDPIDDQDGGQPGGNIRNAYLYDSSIVRLRNLNPGSSSQAQDVFPGAELKYNPGLIDPTHPAWDSSRKPISAVWETLDGKNKFFTVNVHFTSKGGGSSIEGDLRPPANGGIEKRTEQASIVANFTSTLLNTDPSAKIIVSGDFNEFTFVQPLEVFAAESGLTDLDDVVGTKGEERYTYIYDMNCQALDHMFVSGGLKIGAQFEHVHLNTWVSYDEQASDHDPSVARFDVCE

SEQ ID NO: 85 - protein, 590 aa, Stenocarpella maydis
LSISQINGNRFLSPYDGQTLTNISGLVTAKGPTGVFVRSTAPDNDTATSDSAFIYSSSVGSSLNVGDIVTFSAKVAEFRSRGSTYLYLTELTSPADVVVVSRNNTVAPLVVGEDTPYPPTEKFSSLDGGDVYRIPNAVANISAVNPVLDPANYGLDFWESLSAELVTIRNVTVISRPNSYGETWVTGGWPVTGRSARGSLTMTALDSNPEVIKIDEPLDGTSNPASPKIGDKATDITGVVYQQFGFYYIIPLTAYELTTLADGTAPPTTLESTRSCEGITVGDYNVENLSPASANIEGRADHIVNYLGAPDLVFVQEIQDGSGPANDGVVDASATLTALVDAIAAAGNVTYSFVEIAPEDGKDGGQPGGNIRVAYLYRPEVVSLYKPSPGDSTTATRVVAGESGPELTLNPGRIDPANPCWVATRKPLVAAWLAEGATKPFFTVNVHWSSKGGSSSLQGDMRPPVNGVVGNRLAQANVTGQFISEILAIDPSAAVIAAGDFNEFAFVEPLTAFADISGLTELDEVVGIPPEERYTYTFDMNTQALDHMYVSPVLEEGAGYEHIHVNTWAAEEDVVSDHDPSVALFGVCGA

SEQ ID NO: 86 - protein, 596 aa, Acrophialophora fusispora
LTIAEINGNKFISSYNGQAVTNITGLLIAKGPNGVWIRSTTPDDDQATSEAIYVFSSSVGANLTVGDIISLDGKVSEYRSSSNYMYLTEITSPKNVKVVSSGNTVTPLVIGQDTLSPPTVQYSSLDNGDIYNLPNGVANVSAANPVLDPTKYGLDFWESLSGELVTVKKPTAIKTPNQYGDTWVIGDWAVTGRNHHGGVTMSDKDSNPEAIIIGSPLDRTKNPTTSKMGDQFEDITGVVQHAFGFYSILPLTAIKTTTAASAAAPPTTLLSQGKCKAITVGSYNVENLAPNSTHLPKVAAHIVDYLKTPDLIFVQEVQDNSGPTDDGVVSANTTLTTLVDAIHSLSGVTYAFADVDPVSNADGGQPGGNIRQAYLYRPEVVSLYKPNQGGSNDATEVVPGKGNGLAGVPTLSFNPGRIEPGNAAWKASRKPLAAVWKAKGAKRPFYTVNVHWSSKGGGTSLHGDRRPPVNGAVDARMAQANVTGTFIAQILSLDPAANVIAAGDFNEFAFVQPMKTFSAISTMVDLDEAAGIPVEERYTYAYDMNAQALDHMYVSPALAHKKSTRFEHLHVNSWASYDDVVSDHDPSIALFDVCGC

SEQ ID NO: 87 - protein, 598 aa, Chaetomium luteum
LTISEINGNKFISPYSGKSVTNVTGLLIAKGPNGIWIRSTTPDDDKTTSEAVYVFSSSVGINLTVGDIISLDGKVSEYRSSSSYIYLTEITSPKNVHILSSGNTVTPLIIGKDTLSPPTVQYSNLDGGDIYSLPNAVANISEVNPVLDPAKYGLDFWESLSGELVTINKPQAIKTPNEYGDTWVVGDWAVTGKNKHGGLTMSDKDSNPEAIIIGTPLDGTKNPTISKMGDQFEDITGIVQQTFGFYNILPLTALKTTSSASASVSPTFLLSHGKCKALTVGSYNVENMAPTSSHLPKVAAHIVDYLKTPDLMFVQEIQDNSGPTNDGIVSANATITALVKAIKTLSGVTYAWTDIDPVSNEDGGQPGGNIRQAYLYRPEVLSLYEANPGGSNDATEVVPAEGKGKGFGGAPTLSFNPGRIDPANAAWKNSRKPLAAVWKAKGAKRPFYTVNVHWSSKGGGTSLHGDVRPPINGAVEARMAQANVTGSFIAKILALDPTANIIAAGDFNEFSFVQPLKMFSTISKMVDIDEATEVPAEERYTYAYDMNAQALDHIFISPALALSKTTRVDHLHLNSWAAYDDVVSDHDPSIALLDVCGC

SEQ ID NO: 88 - protein, 592 aa, Arthrinium arundinis
LTIGEINGNRFLSPYNGQDVSNVTGIVTAKGPDGLWVRSVRKGCDRRVSDAVYIYGSALATNASISTGDVVVLSGKVSEYRSNKDYLYMTQITSPKVAAILEHGKQVVPKVIGKDTYSPPTVQYTSLDEGDIFAVPNNKSLVSVANPVLEPEKYGLDFWESLSGQLVTVKSPRAIGRPNKYGDTWVVGDWKTSGENGRGGLTTMSMDSNPEGIVIGSPLDGSKNPNDTKLGDTLEDITGVVYQAFGFYRILPLTKVAVVASQEPAMPPPTSLTSDGVCSGLTIGSYNIENFWPGDTAHVQAVAHHIVDYLKTPDLVFLQEVQDDNGATDDGTVSSDLTLSTLAAAIEKASGGIGYNFTYVAPINKKDGGAPGGNIRTAYLFRRDVLTLRDPNPADSTTANEVLSGGALKYNPGLIDPTNAAFTNSRKPLTAAWQTLDGNSTFYTVNVHWGSKGGSSSIHGDARPPVNGGVKDRIAQAAVTANFIAAILAEDPEAHIITSGDFNEYPFVKPITDFESRSKMEDLDVVAGIDPVERYSYLYDMNTQELDHMFVSPALAKTKPQFEHIHVNTWIAYDDMVSDHDPSVAKMNLCKY

SEQ ID NO: 89 - protein, 766 aa, Phialophora geniculata
QSIHAINGKNFLSPYNGALVTNVTGIVTAKASNGLYLRSPKPACDVRIGNGLVVYDSTIGKNESIAVGDTLVLSGKITEYRSTATYLYLTELESPVVQSWVKGETAPKPRVIGTDTMSPPTEHFTGLDNGDVFGIPNDDSRISVVNPELQPDKYGLDFWKSLNGELVTMANPVAISKITTYGETWMVGSWPTTGQNKRGGLTLGDKDGNPEAIIVGAPLDGSRAVDSYRIGDTFQNITGVIRYQFGFYYLLPLTSPVLVSSPSPALPPPTSLISTGECSGLTFGDYNIENFAPSDMAHANDVAAHIVNYLKSPDVLFVQEVQDNSGPTNNGVVDSSVTLSVLASVIANMGGPKYSYTWINPINNADGGQNGGNIRVAYLYNADLVQLSNGSPGGSLDANAVLEDKNGRPTLKYNPGLIDPTNAAWAATRKPLVAQWQTVVGNHVFFTVNVHWSSKGGSSSLQGDPRPPINSPIEKRIQQANVTASFIAQIVESDADARIILAGDLNEFAFVEPVKTFAAVSSMVDLNDAANIPVEERYTYTFGANMQEIDHMFVSPAIANLSPLQEHIHVNTWVSVKDQVSDHDPTVAKLNVCGINIGPNVTSTTTTSTATITSSTSTVTGVVTTTTLTTSTTTSTAAPIASGTALSGRGQFQVTSPGVSSGGSLITAGTWYRGGGTPATYTATPNADGKTFTLATSRGKCAVLADTSFSCGTGITTASSFGFDGTYLTFSGSNVFHAAAVPSGTTQGTIFTSEQAVTLQAIWKPL

SEQ ID NO: 90 - protein, 122 aa, Paenibacillus sp-62212
ETEPTTQQAAGSTSAETITLYFPQDRFPETGKHIKNAIASGESSICTIDRKQAEENRKHSLKGIPTKKGYDRDEWPMAMCAEGGTGADIAYISPSDNRGAGSWVSNQLEKYEDGTKILFIVK

SEQ ID NO: 91 - protein, 118 aa, Paenibacillus sp-62605
NDTSVTTSSTEADVKIVFPSDRFPETAKHIKDAIAAGESPICTIDRDGAEENRKESLKGIATKKGYDRDEWPMAMCAEGGAGADIAYITPSDNRGAGSWVGNQLEKYTDGTRVEFVVE

SEQ ID NO: 92 - protein, 115 aa, Bacillus sp-62738
SETADSKGYDQVVELPADKYPETAAHIKNAIAKGKTDMCTIDRKGAKDRRKQSLAHIPTKKGYDRDEFPMAFCKEGGSGADIEYISPEDNRGAGSYIGNKVENLKDGTRVKIAVN

SEQ ID NO: 93 - protein, 120 aa, Bacillus pumilus
QLEQSKQETTNSSYDKTIHFPSDRYPETAKHIEEAIDEGHSSVCTIDRKHSDEQRDQSLHGIPTKRGYDRDEWPMAMCKEGGTGASVKYISPSDNRGAGSWVGHQLSDDPDGTRIQFIID

SEQ ID NO: 94 - protein, 249 aa, Bacillus horikoshii
VEDGSSTQLANNSTNHEPSIKVREETETNIEENHEFPRTEVPLIRVIDGDTIKVKIDGKEENVRFLLVDTPETSHPRMNGPQPFGPEAKEFMEEFAATGKLELELDVSERDRYGRVLAYVYVNGVSAQEELLKRGLARVAYIYPPNTRYVDHYQALQEKAQADGVGIWSVENYAQDDGFYPEYVEDPDLKESTEKQPVTENCPVKGNISSSGEKIYHVKTGAFYERTIPEECFNTEEEAMKAGYRKSKR

SEQ ID NO: 95 - protein, 245 aa, Bacillus sp-62490
STYEETKPSSTVETDEIEVDETQKEEIIEETSESFIQATVVRVVDGDTVIVKLPNNQEERVRLLLVDTPESVHPTKPVQPFGIESSEFAKQLMYPGKTVELELDINERDKYGRLLAYVWVGEKMLNELLLEKGLARVAYIFAPNTRHVDRFLEIQKKAQQQELGIWSIENYATESGFAEEAVLEKQEPTKLTKACDDPKIKGNHSSSGELIYHIPGGQYYEKTNPEEMFCTEDEALEAGYRKSMR

SEQ ID NO: 96 - protein, 223 aa, Bacillus sp-13390
KESNSKEAVEQRFIQASVVRVVDGDTLIVKLDHKKEERVRLLLIDTPESVHPDKPVQPFGIEASEMVKELMKPGDLIHLELDVSERDKYGRLLAYVWIEDKMVNELLLEKGFARVAYVYAPNTKYVDQFYDIQKQAQERGIGIWSLENYVVDRGFNEEVYLEKDNPSHSDLSCSNPMIKGNHSSRGDFIYHVPEGQYYDQTNAEEMFCTEEEAKAAGYRKSMK

SEQ ID NO: 97 - protein, 210 aa, Jeotgalibacillus sp-13376
DKPERLNAVVTNVVDGDTIDVKTEDGSIERVRLLLIDTPETKHPQMGVQPFGHEASIYTESALLGEKIQLEFDVSERDRYGRVLAYIWHQDELFNQTLIEKGLARVSIYPPDIKYVDEFEKIQEEARKSELGIWSLQNYVTKKGYERKLDQSKDEEIIQPDGCTIKGNINSKGEKIYHDTNSRSYSQTIPEEWFCTIEEAKAAGFRAPRN

SEQ ID NO: 98 - protein, 231 aa, Bacillus sp-62738
STNKQEPSQATTKQESNQTQNKTSNGQQQSYNIEDIAKNYKGQKVVEINGNKADFTQDQLDKVQLKNTNPTWQEFSNLDSKNRVGVATALIGKEIQPKEKRDERLNTKPTGWHQKKLSDGSTLFDRSHLIGYQLTGQNDNPKNLMTGTKDFNRHSMLKYENMVDKEVEKGSYVLYEVKPVFIGDELVARGVQMKAKTVNNNHLDFNVFCFNVQDGVEIDYKDGTSKLVNKQ

SEQ ID NO: 99 - protein, 268 aa, Streptomyces iakyrus
RSLLDLLKPPTQHQEQTSRSGSISQSAALDLYSNQQKQASFDGCAELFPAAKPINVATVPATMNPMALCSDNFAVLYSQTSKTPLIVVERLNASQLQDAKGEERTNQFYPDPRIPKSGRAELSDYRGQHPAVDRGHQSPAADAPNPNAMAQSFALSNMVPQDPTNNRKIWSKVESDVRKFAKRADGNVFVFTGPLFDSGHSTIGENKVWVPTRLFKLVYDASSKRAWAYVLPNAETRIEKPMDYDAFVKSTGLKLLGNLPISGSVGRT

SEQ ID NO: 100 - protein, 245 aa, Streptococcus infantis
SNATPQTQVNQKSQSLDTPSQKLAESVLTDSVKKQIKGTLEWNGSGAFIVNGNKTNLDAKVSSKPYADNKTKTVGGETVPTVANALMSKATRQYKDREETGNGSTSWTPAGWHQVKNLKGTYNHAVDRGHLLGYALIGGLDGFDASTSNPKNIAVQTAWANQARAEDSTGQNYYESLVRKALDQNKRVRYRVTLLYATEEDLVPSASQIEAKSSDGELEFNVVVPNVQKGIQLDYRTGKVTVTKN

SEQ ID NO: 101 - protein, 110 aa, Bacillus sp-62599
ASSYDATLTFPSDKYPYTADHIRDAIAAGQSSICTIDRDGAEQNREESLRGIPTKKGYDRDEWPMAMCEEGGAGADVRYVPSSDNRGSGAWVGNQLSKYPDGTRVKFYVP

SEQ ID NO: 102 - protein, 251 aa, Bacillus akibai
STDENKEDILIETSSAVETDEVEVDEQEHKEESPEESNGTFIQATVVRVVDGDTVIVKLPNNTEERVRLLLIDTPESVHPTKPVQPFGLEASEFAKELMYPGKTVELELDINERDRYGRLLAYVWIGDEMLNELLLENGLARVAYIFAPNTRHVDRFYEIQKKAQQQAIGIWSIENYATEGGFAEEVDLEKQEPSKLANACDDPKIKGNHSSSGDLIYHIPGGQYYEKTNPEEMFCTEEEAKEAGYRKSMR

SEQ ID NO: 103 - protein, 125 aa, Paenibacillus xylanexedens
GGEWPEEIPNPFGGTNKSVDHTITFPSERYPETAKHIKAAIKAGHSDVCTIDRNGAEGNRDLSLKGVPVKKGKDRDEWPMAMCAEGGTGADIQYITPKDNRGAGSWVGNQLSTYPDGTRVKFVVK

SEQ ID NO: 104 - protein, 182 aa, Fictibacillus sp-62719
LPPGTPTKSAAQSQLNALVVKTEGTMTGYSRDLFPHWSSQGGGCDTRQVVLKRDADSFSGNCPVTSGSWYSYYDGITITNPSDLDIDHVVPLAEAWRSGASSWTTDRREAFANDLTGPQLIAVTASSNRSKGDQDPSTWKPTRTAAGCGYAKWWIQTKYNWGLNLQSAEKTSLQSMLNTCTY

SEQ ID NO: 105 - protein, 182 aa, Exiguobacterium sp. NG55
FPPNIPSKADALTKLNALTVKNEGSMTGYSRDIFPHWSSQGSGCNTRHIVLKRDADSVVDQCPVTTGSWYSYYDGLTFTSASDIDIDHVVPLAEAWRSGASSWTTTKRQSFANDLNGPQLIAVSASSNRSKGDQDPSTWQPPRTGARCAYAKMWVETKSRWGLSLQSAEKSALTTAINACSY

SEQ ID NO: 106 - protein, 216 aa, Streptomyces thermoalcalitolerans
CTEDTGGPGTPEKTAAGAALAAVEELPVKGRAPKTGYEREKFGRAWADTDSNGCRTRDDILKRDLEQVRFTDGTCKVSYGVLASDPYSGKEIVFRRGHSQIDIDHVVALSDAWQKGAKYWDASKRIALANDPLNLLAVDARTNRAKGDGDTATWLPPNKAYRCQYVARQVAVKKKYELWVTAAEKAAMKRVLSTCPDQKLPSGGTPTKAPERFRAQ

SEQ ID NO: 107 - protein, 200 aa, Metagenome from environmental sample C
SLPDYASPISTPTSGLATPASDASPSDRKDRTDYDYELVFPSDKYPETALHIHGAIEMGYSDVCTIDRGGAEQNRKESLAGIETRQGYDRDEWPMAMCGEGGAGASVAYIDAGDNRGAGSWVGNQLKEYPDGTRILFIVDKPANLFPAQSPNASSQPADDAEVYYKNCTAVREAGKAPLHKGEPGYAAHLDRDGNGVACE

SEQ ID NO: 108 - protein, 463 aa, Streptomyces davawensis
DATIVINPGTRYGTWEGWGTSLAWWGNVFGTRDDFADLFFTTKSVTYNGTSLPGLGLNIARYNLGACSWNAVNGETMVKSPNIPAFKQIEGFWQDWNNEDPTSSAWDWTADATQRAMLVKATQRGAVTELFANSPMWWMCYNHNPSGAADGGNNLQTWNYRQHASHLAAVALYARTNWGVNFATVDPFNEPASSWWTASGTQEGCHLDPAVQAAVLPYMRSELDKRGLTGVRISASDETNYDTARSTWSSFGSATKALVSQVNVHGYQGTGGRRDLLYTDVVTTSGKKLWNSETGDSDGTGLSMARNLCYDFRWLHPTAWCYWQVMDPSTGWAMIAYDANTLQPTTVQPKYYVMAQFSRHIRPGMTILDTGVSFAAAAYDASARRLVLVAVNTSTSPQTFTFDLSRFTTVTGGSGGLVPRWNTVTGGGDMYRAYTNTYVTGKSVSATFAAGSVQTLQVDGVTT

SEQ ID NO: 109 - protein, 464 aa, Streptomyces avermitilis
DATIAVNPSTTYGKWEGWGTSLAWWANVFGARDDFADLFFTTKSVTYNGRTLPGLGLNIARYNLGACSWNSVSGESMVASANIPAFKQIEGYWQDWNNEDPTSSAWKWTADAAQRTMLVKATARGATTELFANSPMWWMCLNHNPSGASGGGNNLQSWNYRQHASHLAAVALYAKSNWGVNFATVDPFNEPSSSWWTATGTQEGCHMDASVQAAVLPYLRSELDRRGLTGTKISASDETSYDLARTTWGSFGSSTKALVNRVNVHGYQGSGGRRDLLYTDVVTTAGKALWNSETGDSDGTGLTLASNLCLDFRWLHPTAWVYWQVMDPSSGWAMIAYDASTLQPGAVQTKYYVMAQFSRHIRAGMTIVDTGVGYAAAAYDATARRLVIVAVNTSTSAQTLTFDLSRFSTVTGGTGGLVRRWNTVTGGGGDLYAAHSDTYLSGKSLSVPFAAGAVQTLEVDGVTV

SEQ ID NO: 110 - protein, 458 aa, Trichoderma harzianum
DTTLSIDPTSNWGTWEGWGVSLAWWAKAFGNRDDLANVFFTRNNQVINGQNLPGLGFNIARYNAGACSTNTYNGSSMVVSSSIKPSRQVDGYWLDWASTDPASSSWNWNVDANQRAMLQKAKANGANIFELFSNSPMWWMCLNHNPSGSGSSDNLQSWNYQNHAVYLANIAQHAQQNWGIQFQSVEAFNEPSSGWGPTGTQEGCHFAVSTMATVIGYLNTELAQRGLSSFISASDETSYDLAISTWQGLGSSAQNAVKRVNVHGYQGGGGRRDTLYSLVSQAGKRLWNSEYGDADASGKSMYTNLLLDFTWLHPTAWVYWQAIDGSGWGLIVGDNDQLTLSSASTKYFVLAQLTRHIRPGMQILTTPDGNTVAAYDSGSQKLVIVAANWGSAQTITFDLTRAKTAGSNGATVPRWSTQTSGGDQYKSYSDTKINNGKFSVSFSTGQVQTFEISGVVLK

SEQ ID NO: 111 - protein, 541 aa, Ascobolus stictoideus
QTYTLEAEAGTLTGVTVMNEIAGFSGTGYVGGWDEDADTVSLTFTSDATKLYDVKIRYSGPYGSKYTRISYNGATGGDISLPETTEWATVNAGQALLNAGSNTIKLHNNWGWYLIDAVILTPSVPRPPHQVTDALVNTNSNAVTKQLMKFLVSKYHKAYITGQQELHAHQWVEKNVGKSPAILGLDFMDYSPSRVEFGTTSQAVEQAIDFDKRGGIVTFAWHWNAPSGLINTPGSEWWRGFYTEHTTFDVAAALQNTTNANYNLLIRDIDAIAVQLKRLQTAGVPVLWRPLHEAEGGWFWWGAKGPEPAKKLYKILYDRLTNYHKLNNLIWVWNSVAKDWYPGDEIVDVLSFDSYPAQPGDHGPVSAQYNALVELGKDKKLIAATEVGTIPDPDLMQLYESYWSFFVTWEGEFIENGVHNSLEFLKKLYNNSFVLNLDTIQGWKNGAGSSTTTVKSTTTTPTTTIKSTTTTPVTTPTTVKTTTTPTTTATTVKSTTTTAGPTPTAVAGRWQQCGGIGFTGPTTCEAGTTCNVLNPYYSQCL

SEQ ID NO: 112 - protein, 526 aa, Chaetomium virescens
PRDPGATARTFEAEDATLAGTNVDTALSGFTGTGYVTGFDQAADKVTFTVDSASTELYDLSIRVAAIYGDKRTSVVLNGGASSEVYFPAGETWTNVAAGQLLLNQGSNTIDIVSNWGWYLIDSITLTPSTPRPAHQINEAPVNAAADKNAKALYSYLRSIYGKKILSGQQELSLSNWIAQQTGKTPALVSVDLMDYSPSRVERGTVGTAVEEAIQHHNRGGIVSVLWHWNAPTGLYDTEEHRWWSGFYTSATDFDVAAALSSTTNANYTLLIRDIDAIAVQLKRLQSAGVPVLFRPLHEAEGGWFWWGAKGPEPAKKLWGILYDRVTNHHQINNLLWVWNSILPEWYPGDATVDILSADVYAQGNGPMSTQYNQLIELGKDKKMIAAAEVGAAPLPDLLQAYEAHWLWFTVWGDSFINNADWNSLDTLKKVYTSDYVLTLDEIQGWQGSTPSATTTSSTTTPSATTTTTTPSTTATTATPSATTTASPVTYAEHWGQCAGKGWTGPTTCRPPYTCKYQNDWYSQCL

SEQ ID NO: 113 - protein, 452 aa, Preussia aemulans
QTVIYQAEQAKLSGVTVEFSIIKQVVGTGYVEGFDESTDSITFTVESTTAALYDLALTYNGPYGDKYTNVVLNNAAGSQVSLPATTAWTTVPAGQVLLNAGANTIQIQNNWGWYLVDSISLKPAATRGAHQITTKPVNKNANSDAKALLKYLGSIYGKKILSGQQDLSSLDWVTKNVGKTPAVLGLDTMDYSESRKSRGAVSTDVDKAIAFAKKGGIVTFCWHWGAPTGLFDSAAQPWYRGFYTDATDFNIETALKDTTNANYTLLMKDIDTIAVQLKKLQDAGVPVIWRPLHEAEGGWFWWGAKGPEPAKKLWKIMYDRLTNQHGLNNLVWTWNSVAPNWYPGDDTVDIVSADTYSQGDHGPISATYNNLLALTNDTKIIAAAEIGSVMEPAQLQAYQADWVYFCVWSGEFIDGGVWNSLDFLKKVYNDPYVLTLDEIQGWKTARGKPRVS

SEQ ID NO: 114 - protein, 312 aa, Yunnania penicillata
APSTTPVNEKATDAAKNLLSYLVEQAANGVTLSGQQDLESAQWVSDNVGKWPAILGIDFMDYSPSRVEYGAVGSTVPDAISYDSDGGIVTFCWHWGSPSGTYNTTDQPWWSNFYTEATAFDIAAAMDDPDSADYNLLVRDIDAISELLLQLQDLDIPILWRPLHEAEGGWFWWGAKGPEACIALYRLMFDRMTNHHGLNNLLWVWNSVDPSWYPGNDVVDIVSADIYADAGDHSPQEETFASLQSLTGDTKLVALGEVGNIPDPASTGGVADWAYWVTWNGDFIKGEDYNPLEYKKEVFSAENIITRDEVDV

SEQ ID NO: 115 - protein, 327 aa, Myrothecium roridum
GTIENRQWLTYNPVDSAATTEARALLRYIQSQYGWRYLSGQQERAEVQWLKSNIGKTPAIQGSDLIDYSPSRVSYGATSTAVEDAIAFDRQGGIVTFTWHWNAPNCLYNSADQPWYFGFYTKATCFNIQAALAQGSNGADYKLLIRDIDAIAVQLKRLRDAKVPILFRPLHEPDGAWFWWGAKGSGPFKQLWDILYDRLTKYHGLHNMLWVCNTEKSDWYPGNNKCDIATTDVYVNAGDHSVQKSHWDALYGVSGGQRILALGEVGVIPDPERQASENVPWAYWMTWNGYFIRDGNYNSRNFLQSTFSNARVVTLDGTSPLGNWKSS